European Patent Application EP 4 331 606 A1, published March 6, 2024. Title: Treatment or prevention of myopathy by using miR-33b inhibitor. Applicant: Mitsubishi Tanabe Pharma Corporation Kyoto University Osaka University National Institutes of Biomedical Innovation, Health and Nutrition. The sequence listing filed with the application follows.

SEQUENCE LISTING (23 sequences)

SEQ ID NO: 1 - RNA, 20 nt, Homo sapiens
gugcauugcuguugcauugc

SEQ ID NO: 2 - RNA, 21 nt, Homo sapiens
gugcauuguaguugcauugca

SEQ ID NO: 3 - RNA, 21 nt, Homo sapiens
gugcauuguaguugcauugca

SEQ ID NO: 4 - RNA, 96 nt, Homo sapiens
gcgggcggccccgcggugcauugcuguugcauugcacgugugugaggcgggugcagugccucggcagugcagcccggagccggccccuggcaccac

SEQ ID NO: 5 - DNA, 12 bp, Artificial Sequence
  antisense oligonucleotide
aacagcaatgca

SEQ ID NO: 6 - DNA, 16 bp, Artificial Sequence
  antisense oligonucleotide
tgcaacagcaatgcac

SEQ ID NO: 7 - DNA, 12 bp, Artificial Sequence
  antisense oligonucleotide
  modified_base (3)..(3): m5c
  modified_base (11)..(11): m5c
aactacaatgca

SEQ ID NO: 8 - DNA, 12 bp, Artificial Sequence
  antisense oligonucleotide
  modified_base (3)..(3): m5c
  modified_base (11)..(11): m5c
aacagcaatgca

SEQ ID NO: 9 - DNA, 20 bp, Artificial Sequence
  primer
aacagtttgtggcccttttg

SEQ ID NO: 10 - DNA, 20 bp, Artificial Sequence
  primer
agttccaggctggggtactt

SEQ ID NO: 11 - DNA, 12 bp, Artificial Sequence
  antisense oligonucleotide
  modified_base (3)..(3): m5c
  modified_base (11)..(11): m5c
aacaatactacg

SEQ ID NO: 12 - DNA, 20 bp, Artificial Sequence
  primer
tgtttcagcttctccgaggt

SEQ ID NO: 13 - DNA, 21 bp, Artificial Sequence
  primer
ctggactggagcaggactttc

SEQ ID NO: 14 - DNA, 19 bp, Artificial Sequence
  primer
cttctacgcacctggaccg

SEQ ID NO: 15 - DNA, 20 bp, Artificial Sequence
  primer
actgtagtaggcggtgtcgt

SEQ ID NO: 16 - DNA, 22 bp, Artificial Sequence
  primer
gccctccctgcagattatttgg

SEQ ID NO: 17 - DNA, 27 bp, Artificial Sequence
  primer
ctgtccagttgacctttgatactcttc

SEQ ID NO: 18 - DNA, 20 bp, Artificial Sequence
  primer
gagttcgattagccgagtgc

SEQ ID NO: 19 - DNA, 20 bp, Artificial Sequence
  primer
gtcgggttctgattccacat

SEQ ID NO: 20 - DNA, 20 bp, Artificial Sequence
  primer
atggaccgaggaggatgtga

SEQ ID NO: 21 - DNA, 20 bp, Artificial Sequence
  primer
ttgcatctggccttgaggag

SEQ ID NO: 22 - DNA, 20 bp, Artificial Sequence
  primer
aaatggtgaaggtcggtgtg

SEQ ID NO: 23 - DNA, 20 bp, Artificial Sequence
  primer
aatctccactttgccactgc